European Patent Specification EP 3 319 994 B1, published February 7, 2024. Title: MULTISPECIFIC ANTIGEN-BINDING MOLECULES AND USES THEREOF. Applicant: Regeneron Pharmaceuticals, Inc. The sequence listing filed with the application follows.

SEQUENCE LISTING (12 sequences)

SEQ ID NO: 1 - protein, 502 aa, Artificial sequence
  synthetic
MMALGAAGATRVFVAMVAAALGGHPLLGVSATLNSVLNSNAIKNLPPPLGGAAGHPGSAVSAAPGILYPGGNKYQTIDNYQPYPCAEDEECGTDEYCASPTRGGDAGVQICLACRKRRKRCMRHAMCCPGNYCKNGICVSSDQNHFRGEIEETITESFGNDHSTLDGYSRRTTLSSKMYHTKGQEGSVCLRSSDCASGLCCARHFWSKICKPVLKEGQVCTKHRRKGSHGLEIFQRCYCGEGLSCRIQKDHHQASNSSRLHTCQRHGPGEPRGPTIKPCPPCKCPAPNLLGGPSVFIFPPKIKDVLMISLSPIVTCVVVDVSEDDPDVQISWFVNNVEVHTAQTQTHREDYNSTLRVVSALPIQHQDWMSGKEFKCKVNNKDLPAPIERTISKPKGSVRAPQVYVLPPPEEEMTKKQVTLTCMVTDFMPEDIYVEWTNNGKTELNYKNTEPVLDSDGSYFMYSKLRVEKKNWVERNSYSCSVVHEGLHNHHTTKSFSRTPGK

SEQ ID NO: 2 - protein, 496 aa, Artificial sequence
  synthetic
MMALGAAGATRVFVAMVAAALGGHPLLGVSATLNSVLNSNAIKNLPPPLGGAAGHPGSAVSAAPGILYPGGNKYQTIDNYQPYPCAEDEECGTDEYCASPTRGGDAGVQICLACRKRRKRCMRHAMCCPGNYCKNGICVSSDQNHFRGEIEETITESFGNDHSTLDGYSRRTTLSSKMYHTKGQEGSVCLRSSDCASGLCCARHFWSKICKPVLKEGQVCTKHRRKGSHGLEIFQRCYCGEGLSCRIQKDHHQASNSSRLHTCQRHGPGDKTHTCPPCPAPELLGGPSVFLFPPKPKDTLMISRTPEVTCVVVDVSHEDPEVKFNWYVDGVEVHNAKTKPREEQYNSTYRVVSVLTVLHQDWLNGKEYKCKVSNKALPAPIEKTISKAKGQPREPQVYTLPPSRDELTKNQVSLTCLVKGFYPSDIAVEWESNGQPENNYKTTPPVLDSDGSFFLYSKLTVDKSRWQQGNVFSCSVMHEALHNHYTQKSLSLSPGK

SEQ ID NO: 3 - protein, 122 aa, Artificial sequence
  synthetic
EVQLVESGGGVVQPGRSLRLSCVASGFTFSDYGMHWVRQAPGKGLEWVAVIWYDGSIKYFRDSVKGRFTISRDNSKNTLYLQMNSLRVEDTAHYYCAKESSSWYFYHGLDVWGQGTMVTVSS

SEQ ID NO: 4 - protein, 114 aa, Artificial sequence
  synthetic
EIVMTQSPLSLPVSPGEPASISCRSNQSLLHSNGNNYLAWYLQKPGQSPHLLIYLGSNRASGVPDRFSGSGSGTDFTLKISRVEAGDVGTYFCMQSLQAPPFTFGPGTKVEIKR

SEQ ID NO: 5 - protein, 692 aa, Artificial sequence
  synthetic
MGTVSSRRSWWPLPLLLLLLLLLGPAGARAQEDEDGDYEELVLALRSEEDGLAEAPEHGTTATFHRCAKDPWRLPGTYVVVLKEETHLSQSERTARRLQAQAARRGYLTKILHVFHGLLPGFLVKMSGDLLELALKLPHVDYIEEDSSVFAQSIPWNLERITPPRYRADEYQPPDGGSLVEVYLLDTSIQSDHREIEGRVMVTDFENVPEEDGTRFHRQASKCDSHGTHLAGVVSGRDAGVAKGASMRSLRVLNCQGKGTVSGTLIGLEFIRKSQLVQPVGPLVVLLPLAGGYSRVLNAACQRLARAGVVLVTAAGNFRDDACLYSPASAPEVITVGATNAQDQPVTLGTLGTNFGRCVDLFAPGEDIIGASSDCSTCFVSQSGTSQAAAHVAGIAAMMLSAEPELTLAELRQRLIHFSAKDVINEAWFPEDQRVLTPNLVAALPPSTHGAGWQLFCRTVWSAHSGPTRMATAVARCAPDEELLSCSSFSRSGKRRGERMEAQGGKLVCRAHNAFGGEGVYAIARCCLLPQANCSVHTAPPAEASMGTRVHCHQQGHVLTGCSSHWEVEDLGTHKPPVLRPRGQPNQCVGHREASIHASCCHAPGLECKVKEHGIPAPQEQVTVACEEGWTLTGCSALPGTSHVLGAYAVDNTCVVRSRDVSTTGSTSEGAVTAVAICCRSRHLAQASQELQ

SEQ ID NO: 6 - protein, 15 aa, Artificial sequence
  synthetic
GGGGSGGGGSGGGGS

SEQ ID NO: 7 - protein, 662 aa, Homo sapiens
QEDEDGDYEELVLALRSEEDGLAEAPEHGTTATFHRCAKDPWRLPGTYVVVLKEETHLSQSERTARRLQAQAARRGYLTKILHVFHGLLPGFLVKMSGDLLELALKLPHVDYIEEDSSVFAQSIPWNLERITPPRYRADEYQPPDGGSLVEVYLLDTSIQSDHREIEGRVMVTDFENVPEEDGTRFHRQASKCDSHGTHLAGVVSGRDAGVAKGASMRSLRVLNCQGKGTVSGTLIGLEFIRKSQLVQPVGPLVVLLPLAGGYSRVLNAACQRLARAGVVLVTAAGNFRDDACLYSPASAPEVITVGATNAQDQPVTLGTLGTNFGRCVDLFAPGEDIIGASSDCSTCFVSQSGTSQAAAHVAGIAAMMLSAEPELTLAELRQRLIHFSAKDVINEAWFPEDQRVLTPNLVAALPPSTHGAGWQLFCRTVWSAHSGPTRMATAVARCAPDEELLSCSSFSRSGKRRGERMEAQGGKLVCRAHNAFGGEGVYAIARCCLLPQANCSVHTAPPAEASMGTRVHCHQQGHVLTGCSSHWEVEDLGTHKPPVLRPRGQPNQCVGHREASIHASCCHAPGLECKVKEHGIPAPQEQVTVACEEGWTLTGCSALPGTSHVLGAYAVDNTCVVRSRDVSTTGSTSEGAVTAVAICCRSRHLAQASQELQ

SEQ ID NO: 8 - protein, 267 aa, Homo sapiens
EAWFPEDQRVLTPNLVAALPPSTHGAGWQLFCRTVWSAHSGPTRMATAVARCAPDEELLSCSSFSRSGKRRGERMEAQGGKLVCRAHNAFGGEGVYAIARCCLLPQANCSVHTAPPAEASMGTRVHCHQQGHVLTGCSSHWEVEDLGTHKPPVLRPRGQPNQCVGHREASIHASCCHAPGLECKVKEHGIPAPQEQVTVACEEGWTLTGCSALPGTSHVLGAYAVDNTCVVRSRDVSTTGSTSEGAVTAVAICCRSRHLAQASQELQ

SEQ ID NO: 9 - protein, 243 aa, Homo sapiens
GAGWQLFCRTVWSAHSGPTRMATAVARCAPDEELLSCSSFSRSGKRRGERMEAQGGKLVCRAHNAFGGEGVYAIARCCLLPQANCSVHTAPPAEASMGTRVHCHQQGHVLTGCSSHWEVEDLGTHKPPVLRPRGQPNQCVGHREASIHASCCHAPGLECKVKEHGIPAPQEQVTVACEEGWTLTGCSALPGTSHVLGAYAVDNTCVVRSRDVSTTGSTSEGAVTAVAICCRSRHLAQASQELQ

SEQ ID NO: 10 - protein, 399 aa, Homo sapiens
MGEPGQSPSPRSSHGSPPTLSTLTLLLLLCGHAHSQCKILRCNAEYVSSTLSLRGGGSSGALRGGGGGGRGGGVGSGGLCRALRSYALCTRRTARTCRGDLAFHSAVHGIEDLMIQHNCSRQGPTAPPPPRGPALPGAGSGLPAPDPCDYEGRFSRLHGRPPGFLHCASFGDPHVRSFHHHFHTCRVQGAWPLLDNDFLFVQATSSPMALGANATATRKLTIIFKNMQECIDQKVYQAEVDNLPVAFEDGSINGGDRPGGSSLSIQTANPGNHVEIQAAYIGTTIIIRQTAGQLSFSIKVAEDVAMAFSAEQDLQLCVGGCPPSQRLSRSERNRRGAITIDTARRLCKEGLPVEDAYFHSCVFDVLISGDPNFTVAAQAALEDARAFLPDLEKLHLFPS

SEQ ID NO: 11 - protein, 622 aa, Homo sapiens
MKENVASATVFTLLLFLNTCLLNGQLPPGKPEIFKCRSPNKETFTCWWRPGTDGGLPTNYSLTYHREGETLMHECPDYITGGPNSCHFGKQYTSMWRTYIMMVNATNQMGSSFSDELYVDVTYIVQPDPPLELAVEVKQPEDRKPYLWIKWSPPTLIDLKTGWFTLLYEIRLKPEKAAEWEIHFAGQQTEFKILSLHPGQKYLVQVRCKPDHGYWSAWSPATFIQIPSDFTMNDTTVWISVAVLSAVICLIIVWAVALKGYSMVTCIFPPVPGPKIKGFDAHLLEKGKSEELLSALGCQDFPPTSDYEDLLVEYLEVDDSEDQHLMSVHSKEHPSQGMKPTYLDPDTDSGRGSCDSPSLLSEKCEEPQANPSTFYDPEVIEKPENPETTHTWDPQCISMEGKIPYFHAGGSKCSTWPLPQPSQHNPRSSYHNITDVCELAVGPAGAPATLLNEAGKDALKSSQTIKSREEGKATQQREVESFHSETDQDTPWLLPQEKTPFGSAKPLDYVEIHKVNKDGALSLLPKQRENSGKPKKPGTPENNKEYAKVSGVMDNNILVLVPDPHAKNVACFEESAKEAPPSLEQNQAEKALANFTATSSKCRLQLGGLDYLDPACFTHSFH

SEQ ID NO: 12 - protein, 21 aa, Homo sapiens
DAHLLEKGKSEELLSALGCQD